European Patent Specification EP 4 092 042 B1, published February 12, 2025. Title: Novel branched-chain amino acid permease variant and a method for producing L-valine using the same. Applicant: CJ CheilJedang Corporation. The sequence listing filed with the application follows.

SEQUENCE LISTING (10 sequences)

SEQ ID NO: 1 - protein, 426 aa, Artificial Sequence
  branched-chain amino acid permease variant
MSKKSVLITSLMLFSMFFGAGNLIFPPMLGLSAGTNYLPAILGFLATSVLLPVLAIIAVVLSGENVKDMASRGGKIFGLVFPIAAYLSIGAFYALPRTGAVSYSTAVGVDNTLYSGLFNFVFFAVALALSWNPNGIADKLGKWLTPALLTLIVVLVVLSVAKLDGTPGEPSSAYAQQPAGAGLLEGYMTMDAIAALAFGIVVISAFKYQKVNKVRTATVVSAFIAGILLALVYLGLGSIGQVVNGEFADGTAILNYAALSTMGQAGRIMFVAILILACMTTAVGLISATSEFFNSLLPGVKYHVWATVFALISFGVATMGLDTVLAVAAPVISFIYPSAITLVFLSLIEPLLFRLKWTYLFGIWTAVVWALFMSIPALNPFIEWAPLHSMSLGWVVPVLVASAIGLAIDWNKKGAQSVAEKESISV

SEQ ID NO: 2 - DNA, 1281 bp, Artificial Sequence
  branched-chain amino acid permease variant coding gene
atgagtaaaaagtctgtcctgattacttctttgatgctgttttccatgttcttcggagctggaaacctcatcttcccgccgatgcttggattgtcggcaggaaccaactatctaccagctatcttaggatttctagcaacgagtgttctgctcccggtgctggcgattatcgcggtggtgttgtcgggagaaaatgtcaaggacatggcttctcgtggcggtaagatctttggcctggtgtttcctattgctgcctatttgtccatcggtgcgttttacgcgctgccgaggactggggcggtgagctattcgacggcggttggcgtcgataatacgctttattcgggcttgtttaactttgtgttttttgcggtggcactggcgttgtcgtggaatccgaatggcattgcagacaagttgggtaagtggctcacgccagcgttgctcacgttgattgtggtgctggtggtgttgtcggtagccaagttggatggcacgccaggtgagccaagtagtgcgtatgcgcagcagcctgcgggggcgggtttgcttgagggctacatgacgatggatgcgattgctgcgttggcgtttggcatcgtggtgatttctgcgttcaagtaccaaaaggttaacaaggtccgcacggcaactgtcgtgtcggcgttcattgccggaattttgttggcgctggtttatcttggtttgggctcaatcggtcaagtagtaaacggtgagttcgctgatggcaccgcaattttgaactacgctgcactgtccacgatgggtcaggctggtcgcatcatgttcgtggccattttgatccttgcatgtatgaccaccgcagttggtctgatcagtgcgacgtctgagtttttcaattcgctgctgccaggtgtcaagtaccacgtctgggccactgttttcgcgctgatttcctttggcgttgccacgatgggattggatacggtgttggccgttgcggctccagtgattagtttcatttacccatcggccatcaccttggtgttcttgtcgctcatcgagcccctgctgttccgtctcaagtggacctacctattcggcatttggactgcagttgtgtgggcgctgttcatgtctatccctgcgctgaatccattcatcgaatgggcgccgctgcacagcatgtctttgggttgggttgtcccagttctcgtggcctctgccatcggtttggctattgattggaacaagaaaggtgcccagtctgttgcagagaaggaatccatttccgtctaa

SEQ ID NO: 3 - protein, 426 aa, Artificial Sequence
  Wild-type branched-chain amino acid permease
MSKKSVLITSLMLFSMFFGAGNLIFPPMLGLSAGTNYLPAILGFLATSVLLPVLAIIAVVLSGENVKDMASRGGKIFGLVFPIAAYLSIGAFYALPRTGAVSYSTAVGVDNALYSGLFNFVFFAVALALSWNPNGIADKLGKWLTPALLTLIVVLVVLSVAKLDGTPGEPSSAYAQQPAGAGLLEGYMTMDAIAALAFGIVVISAFKYQKVNKVRTATVVSAFIAGILLALVYLGLGSIGQVVNGEFADGTAILNYAALSTMGQAGRIMFVAILILACMTTAVGLISATSEFFNSLLPGVKYHVWATVFALISFGVATMGLDTVLAVAAPVISFIYPSAITLVFLSLIEPLLFRLKWTYLFGIWTAVVWALFMSIPALNPFIEWAPLHSMSLGWVVPVLVASAIGLAIDWNKKGAQSVAEKESISV

SEQ ID NO: 4 - DNA, 1281 bp, Artificial Sequence
  Wild-type branched-chain amino acid permease coding gene
atgagtaaaaagtctgtcctgattacttctttgatgctgttttccatgttcttcggagctggaaacctcatcttcccgccgatgcttggattgtcggcaggaaccaactatctaccagctatcttaggatttctagcaacgagtgttctgctcccggtgctggcgattatcgcggtggtgttgtcgggagaaaatgtcaaggacatggcttctcgtggcggtaagatctttggcctggtgtttcctattgctgcctatttgtccatcggtgcgttttacgcgctgccgaggactggggcggtgagctattcgacggcggttggcgtcgataatgcgctttattcgggcttgtttaactttgtgttttttgcggtggcactggcgttgtcgtggaatccgaatggcattgcagacaagttgggtaagtggctcacgccagcgttgctcacgttgattgtggtgctggtggtgttgtcggtagccaagttggatggcacgccaggtgagccaagtagtgcgtatgcgcagcagcctgcgggggcgggtttgcttgagggctacatgacgatggatgcgattgctgcgttggcgtttggcatcgtggtgatttctgcgttcaagtaccaaaaggttaacaaggtccgcacggcaactgtcgtgtcggcgttcattgccggaattttgttggcgctggtttatcttggtttgggctcaatcggtcaagtagtaaacggtgagttcgctgatggcaccgcaattttgaactacgctgcactgtccacgatgggtcaggctggtcgcatcatgttcgtggccattttgatccttgcatgtatgaccaccgcagttggtctgatcagtgcgacgtctgagtttttcaattcgctgctgccaggtgtcaagtaccacgtctgggccactgttttcgcgctgatttcctttggcgttgccacgatgggattggatacggtgttggccgttgcggctccagtgattagtttcatttacccatcggccatcaccttggtgttcttgtcgctcatcgagcccctgctgttccgtctcaagtggacctacctattcggcatttggactgcagttgtgtgggcgctgttcatgtctatccctgcgctgaatccattcatcgaatgggcgccgctgcacagcatgtctttgggttgggttgtcccagttctcgtggcctctgccatcggtttggctattgattggaacaagaaaggtgcccagtctgttgcagagaaggaatccatttccgtctaa

SEQ ID NO: 5 - DNA, 40 bp, Artificial Sequence
  brnQ_1F
tgaattcgagctcggtacccttgatgtggttggacttcgc

SEQ ID NO: 6 - DNA, 33 bp, Artificial Sequence
  brnQ_2R
aagcccgaataaagcgtattatcgacgccaacc

SEQ ID NO: 7 - DNA, 33 bp, Artificial Sequence
  brnQ_3F
ggttggcgtcgataatacgctttattcgggctt

SEQ ID NO: 8 - DNA, 40 bp, Artificial Sequence
  brnQ_4R
gtcgactctagaggatccccgcactgatcagaccaactgc

SEQ ID NO: 9 - DNA, 20 bp, Artificial Sequence
  brnQ_5F
ttgatgtggttggacttcgc

SEQ ID NO: 10 - DNA, 20 bp, Artificial Sequence
  brnQ_6R
gcactgatcagaccaactgc